European Patent Application EP 4 219 524 A2, published August 2, 2023. Title: NOVEL PEPTIDES AND COMBINATION OF PEPTIDES FOR USE IN IMMUNOTHERAPY AGAINST AML AND OTHER CANCERS. Applicant: immatics biotechnologies GmbH. The sequence listing filed with the application follows.

SEQUENCE LISTING (200 sequences)

SEQ ID NO: 1 - protein, 9 aa, Homo sapiens
LLDSAVYYL

SEQ ID NO: 2 - protein, 9 aa, Homo sapiens
VLLKAVAQA

SEQ ID NO: 3 - protein, 11 aa, Homo sapiens
ALYDKTKRIFL

SEQ ID NO: 4 - protein, 9 aa, Homo sapiens
FLPDAFVTM

SEQ ID NO: 5 - protein, 10 aa, Homo sapiens
FLYYEDLVSC

SEQ ID NO: 6 - protein, 9 aa, Homo sapiens
GLAEVLLAA

SEQ ID NO: 7 - protein, 9 aa, Homo sapiens
LLWGDIMEL

SEQ ID NO: 8 - protein, 10 aa, Homo sapiens
LLWPGAALLV

SEQ ID NO: 9 - protein, 9 aa, Homo sapiens
SLLAYLEQA

SEQ ID NO: 10 - protein, 9 aa, Homo sapiens
VILDPVHSV

SEQ ID NO: 11 - protein, 9 aa, Homo sapiens
ILTQIDHIL

SEQ ID NO: 12 - protein, 9 aa, Homo sapiens
ALIESNTAL

SEQ ID NO: 13 - protein, 9 aa, Homo sapiens
ALVPGVTQV

SEQ ID NO: 14 - protein, 9 aa, Homo sapiens
ALWWGTITL

SEQ ID NO: 15 - protein, 11 aa, Homo sapiens
FIDEEVEDMYL

SEQ ID NO: 16 - protein, 9 aa, Homo sapiens
FLDTQAPSL

SEQ ID NO: 17 - protein, 9 aa, Homo sapiens
FLLGLSEQL

SEQ ID NO: 18 - protein, 9 aa, Homo sapiens
GIIEENWQL

SEQ ID NO: 19 - protein, 9 aa, Homo sapiens
GIVEYLSLV

SEQ ID NO: 20 - protein, 9 aa, Homo sapiens
GLDAFLLEL

SEQ ID NO: 21 - protein, 9 aa, Homo sapiens
GLFHGTELL

SEQ ID NO: 22 - protein, 10 aa, Homo sapiens
GLLQLDTAFV

SEQ ID NO: 23 - protein, 10 aa, Homo sapiens
GLLQPPVRIV

SEQ ID NO: 24 - protein, 9 aa, Homo sapiens
GLVELLNRV

SEQ ID NO: 25 - protein, 11 aa, Homo sapiens
GVEGSLIVEKI

SEQ ID NO: 26 - protein, 13 aa, Homo sapiens
NAGVEGSLIVEKI

SEQ ID NO: 27 - protein, 9 aa, Homo sapiens
KANPALYVL

SEQ ID NO: 28 - protein, 9 aa, Homo sapiens
LLDQMETPL

SEQ ID NO: 29 - protein, 9 aa, Homo sapiens
RLGPSVVGL

SEQ ID NO: 30 - protein, 9 aa, Homo sapiens
SIISDSSAL

SEQ ID NO: 31 - protein, 9 aa, Homo sapiens
SLFVFIPMV

SEQ ID NO: 32 - protein, 9 aa, Homo sapiens
SLSDRSWHL

SEQ ID NO: 33 - protein, 11 aa, Homo sapiens
TIMNQEKLAKL

SEQ ID NO: 34 - protein, 9 aa, Homo sapiens
TLSPWSFLI

SEQ ID NO: 35 - protein, 11 aa, Homo sapiens
VLFEHAVGYAL

SEQ ID NO: 36 - protein, 9 aa, Homo sapiens
VLGPSPSSV

SEQ ID NO: 37 - protein, 11 aa, Homo sapiens
VVAPAPVVEAV

SEQ ID NO: 38 - protein, 9 aa, Homo sapiens
AAIASTPTL

SEQ ID NO: 39 - protein, 9 aa, Homo sapiens
AIFAGTMQL

SEQ ID NO: 40 - protein, 12 aa, Homo sapiens
ALAAGGYDVEKN

SEQ ID NO: 41 - protein, 10 aa, Homo sapiens
ALFILPFVSV

SEQ ID NO: 42 - protein, 9 aa, Homo sapiens
ALTTYTIEV

SEQ ID NO: 43 - protein, 9 aa, Homo sapiens
AMLDFVSSL

SEQ ID NO: 44 - protein, 11 aa, Homo sapiens
FAVDNVGNRTL

SEQ ID NO: 45 - protein, 9 aa, Homo sapiens
FLFTDVLLM

SEQ ID NO: 46 - protein, 9 aa, Homo sapiens
GLDQYLQEV

SEQ ID NO: 47 - protein, 9 aa, Homo sapiens
GLISPNVQL

SEQ ID NO: 48 - protein, 9 aa, Homo sapiens
IAIEALTQL

SEQ ID NO: 49 - protein, 9 aa, Homo sapiens
IIDDNHAIV

SEQ ID NO: 50 - protein, 9 aa, Homo sapiens
IIWATSLLL

SEQ ID NO: 51 - protein, 9 aa, Homo sapiens
SLLSSSLNV

SEQ ID NO: 52 - protein, 9 aa, Homo sapiens
IVDPVDSTL

SEQ ID NO: 53 - protein, 9 aa, Homo sapiens
KAFLGELTL

SEQ ID NO: 54 - protein, 9 aa, Homo sapiens
KLPEFLVQL

SEQ ID NO: 55 - protein, 9 aa, Homo sapiens
KTLDLINKL

SEQ ID NO: 56 - protein, 9 aa, Homo sapiens
LANPTTSAL

SEQ ID NO: 57 - protein, 12 aa, Homo sapiens
LLDFGSLSNLQV

SEQ ID NO: 58 - protein, 9 aa, Homo sapiens
LLLATLQEA

SEQ ID NO: 59 - protein, 11 aa, Homo sapiens
LSVPEGAIVSL

SEQ ID NO: 60 - protein, 9 aa, Homo sapiens
NLLNVLEYL

SEQ ID NO: 61 - protein, 11 aa, Homo sapiens
FLLPGVLLSEA

SEQ ID NO: 62 - protein, 9 aa, Homo sapiens
RLLFNLSEV

SEQ ID NO: 63 - protein, 9 aa, Homo sapiens
RLNDTIQLL

SEQ ID NO: 64 - protein, 9 aa, Homo sapiens
SLANIKIWV

SEQ ID NO: 65 - protein, 11 aa, Homo sapiens
SLEEQLSALTL

SEQ ID NO: 66 - protein, 10 aa, Homo sapiens
SLKNEVGGLV

SEQ ID NO: 67 - protein, 9 aa, Homo sapiens
SLQDRVIAL

SEQ ID NO: 68 - protein, 10 aa, Homo sapiens
TGITTPVASV

SEQ ID NO: 69 - protein, 9 aa, Homo sapiens
TIIGLVRVI

SEQ ID NO: 70 - protein, 9 aa, Homo sapiens
TLTDSNAQL

SEQ ID NO: 71 - protein, 9 aa, Homo sapiens
TLTSSLATV

SEQ ID NO: 72 - protein, 11 aa, Homo sapiens
VAFPSGDASSL

SEQ ID NO: 73 - protein, 9 aa, Homo sapiens
VAIPDVDPL

SEQ ID NO: 74 - protein, 9 aa, Homo sapiens
VANPVLYVL

SEQ ID NO: 75 - protein, 9 aa, Homo sapiens
VLAPLGFTL

SEQ ID NO: 76 - protein, 9 aa, Homo sapiens
VLLSPVPEL

SEQ ID NO: 77 - protein, 9 aa, Homo sapiens
VLNMKPPEI

SEQ ID NO: 78 - protein, 9 aa, Homo sapiens
VLSEVECHL

SEQ ID NO: 79 - protein, 10 aa, Homo sapiens
YLMDPDTFTF

SEQ ID NO: 80 - protein, 9 aa, Homo sapiens
YLTEALQSI

SEQ ID NO: 81 - protein, 9 aa, Homo sapiens
YVTEELPQL

SEQ ID NO: 82 - protein, 9 aa, Homo sapiens
LLPDNFIAA

SEQ ID NO: 83 - protein, 10 aa, Homo sapiens
GLGAGVAEAV

SEQ ID NO: 84 - protein, 9 aa, Homo sapiens
GLLGSVLTI

SEQ ID NO: 85 - protein, 9 aa, Homo sapiens
GLVPFGLYL

SEQ ID NO: 86 - protein, 10 aa, Homo sapiens
HLLGDPMANV

SEQ ID NO: 87 - protein, 9 aa, Homo sapiens
ILKPFGNSI

SEQ ID NO: 88 - protein, 9 aa, Homo sapiens
LALNFGSTL

SEQ ID NO: 89 - protein, 11 aa, Homo sapiens
LLESPVDGWQV

SEQ ID NO: 90 - protein, 9 aa, Homo sapiens
LLLDTVTSI

SEQ ID NO: 91 - protein, 9 aa, Homo sapiens
RLAHYIDRV

SEQ ID NO: 92 - protein, 9 aa, Homo sapiens
RLWDIQHQL

SEQ ID NO: 93 - protein, 9 aa, Homo sapiens
SLINDVLAE

SEQ ID NO: 94 - protein, 9 aa, Homo sapiens
SLLEFAQYL

SEQ ID NO: 95 - protein, 9 aa, Homo sapiens
SVAEINVLI

SEQ ID NO: 96 - protein, 9 aa, Homo sapiens
TLLASYVFL

SEQ ID NO: 97 - protein, 9 aa, Homo sapiens
TIMTGVIGV

SEQ ID NO: 98 - protein, 9 aa, Homo sapiens
TQFGFLMEV

SEQ ID NO: 99 - protein, 10 aa, Homo sapiens
YLAPFSLSNY

SEQ ID NO: 100 - protein, 14 aa, Homo sapiens
AAPAVLGEVDTSLV

SEQ ID NO: 101 - protein, 13 aa, Homo sapiens
AINKDPEAPIFQV

SEQ ID NO: 102 - protein, 9 aa, Homo sapiens
ALAQGAERV

SEQ ID NO: 103 - protein, 9 aa, Homo sapiens
ALGDFGIRL

SEQ ID NO: 104 - protein, 9 aa, Homo sapiens
ALIPETTTL

SEQ ID NO: 105 - protein, 9 aa, Homo sapiens
GVFALVTAV

SEQ ID NO: 106 - protein, 11 aa, Homo sapiens
ALLEELERSTL

SEQ ID NO: 107 - protein, 9 aa, Homo sapiens
ALLGMLPLL

SEQ ID NO: 108 - protein, 12 aa, Homo sapiens
ELEMNSDLKAQL

SEQ ID NO: 109 - protein, 10 aa, Homo sapiens
GLLAVPLLAA

SEQ ID NO: 110 - protein, 13 aa, Homo sapiens
GLTHTAVVPLDLV

SEQ ID NO: 111 - protein, 14 aa, Homo sapiens
GVEPAADGKGVVVV

SEQ ID NO: 112 - protein, 9 aa, Homo sapiens
ILRDALNQA

SEQ ID NO: 113 - protein, 9 aa, Homo sapiens
NLQSEVEGV

SEQ ID NO: 114 - protein, 9 aa, Homo sapiens
RLAQEAAQV

SEQ ID NO: 115 - protein, 9 aa, Homo sapiens
SLPDLTTPL

SEQ ID NO: 116 - protein, 9 aa, Homo sapiens
TILEILPEL

SEQ ID NO: 117 - protein, 9 aa, Homo sapiens
TILPTILFL

SEQ ID NO: 118 - protein, 9 aa, Homo sapiens
TLLTVLTQA

SEQ ID NO: 119 - protein, 9 aa, Homo sapiens
TLTDELAAL

SEQ ID NO: 120 - protein, 9 aa, Homo sapiens
VIQDLVVSV

SEQ ID NO: 121 - protein, 9 aa, Homo sapiens
VLQAGQYGV

SEQ ID NO: 122 - protein, 9 aa, Homo sapiens
VLYLEEVLL

SEQ ID NO: 123 - protein, 9 aa, Homo sapiens
YTVKINPTL

SEQ ID NO: 124 - protein, 9 aa, Homo sapiens
GLPELVIQL

SEQ ID NO: 125 - protein, 9 aa, Homo sapiens
GLFGYLVFL

SEQ ID NO: 126 - protein, 10 aa, Homo sapiens
GLLPQQIQAV

SEQ ID NO: 127 - protein, 9 aa, Homo sapiens
KIISALPQL

SEQ ID NO: 128 - protein, 9 aa, Homo sapiens
NLSTKTEAV

SEQ ID NO: 129 - protein, 9 aa, Homo sapiens
RMAVLNEQV

SEQ ID NO: 130 - protein, 10 aa, Homo sapiens
GVLGNALEGV

SEQ ID NO: 131 - protein, 10 aa, Homo sapiens
SLFSGSLEPV

SEQ ID NO: 132 - protein, 9 aa, Homo sapiens
SLYPVLNFL

SEQ ID NO: 133 - protein, 9 aa, Homo sapiens
TVIGTLLFL

SEQ ID NO: 134 - protein, 10 aa, Homo sapiens
AAGAGLPESV

SEQ ID NO: 135 - protein, 9 aa, Homo sapiens
GIIDRIFQA

SEQ ID NO: 136 - protein, 9 aa, Homo sapiens
GLSSIETLL

SEQ ID NO: 137 - protein, 9 aa, Homo sapiens
ILAPLAWDL

SEQ ID NO: 138 - protein, 9 aa, Homo sapiens
ILSDNLRQV

SEQ ID NO: 139 - protein, 9 aa, Homo sapiens
NLIIFSPSV

SEQ ID NO: 140 - protein, 9 aa, Homo sapiens
YIPDFLTLL

SEQ ID NO: 141 - protein, 12 aa, Homo sapiens
GLLPPLRIPELL

SEQ ID NO: 142 - protein, 10 aa, Homo sapiens
GLSDGYGFTT

SEQ ID NO: 143 - protein, 9 aa, Homo sapiens
YLLPHILVY

SEQ ID NO: 144 - protein, 9 aa, Homo sapiens
GLFMGLVLV

SEQ ID NO: 145 - protein, 9 aa, Homo sapiens
VLLPLIFTI

SEQ ID NO: 146 - protein, 9 aa, Homo sapiens
ALDTRVVEL

SEQ ID NO: 147 - protein, 9 aa, Homo sapiens
FALPILNAL

SEQ ID NO: 148 - protein, 9 aa, Homo sapiens
FLYFEDHGL

SEQ ID NO: 149 - protein, 9 aa, Homo sapiens
GLAEILVLV

SEQ ID NO: 150 - protein, 9 aa, Homo sapiens
GLFGVLNEI

SEQ ID NO: 151 - protein, 10 aa, Homo sapiens
GLLPFPEVTL

SEQ ID NO: 152 - protein, 9 aa, Homo sapiens
GLSNHIAAL

SEQ ID NO: 153 - protein, 9 aa, Homo sapiens
GLYTGQLAL

SEQ ID NO: 154 - protein, 9 aa, Homo sapiens
IIADNIIFL

SEQ ID NO: 155 - protein, 9 aa, Homo sapiens
ILDLIQVFV

SEQ ID NO: 156 - protein, 9 aa, Homo sapiens
ILMPELASL

SEQ ID NO: 157 - protein, 9 aa, Homo sapiens
ILTETQQGL

SEQ ID NO: 158 - protein, 9 aa, Homo sapiens
LLLGGTALA

SEQ ID NO: 159 - protein, 9 aa, Homo sapiens
LLPLAPAAA

SEQ ID NO: 160 - protein, 9 aa, Homo sapiens
RLVPFLVFV

SEQ ID NO: 161 - protein, 9 aa, Homo sapiens
SLIGIAIAL

SEQ ID NO: 162 - protein, 9 aa, Homo sapiens
SLLDFLTFA

SEQ ID NO: 163 - protein, 9 aa, Homo sapiens
SLMIDLIEV

SEQ ID NO: 164 - protein, 10 aa, Homo sapiens
SLNPQEDVEF

SEQ ID NO: 165 - protein, 9 aa, Homo sapiens
SLVDRVAAA

SEQ ID NO: 166 - protein, 9 aa, Homo sapiens
VLFPLNLQL

SEQ ID NO: 167 - protein, 9 aa, Homo sapiens
VLLDVALGL

SEQ ID NO: 168 - protein, 9 aa, Homo sapiens
VLLFETALL

SEQ ID NO: 169 - protein, 9 aa, Homo sapiens
VLQDPIWLL

SEQ ID NO: 170 - protein, 9 aa, Homo sapiens
IVTEVAVGV

SEQ ID NO: 171 - protein, 9 aa, Homo sapiens
KLLKQVDFL

SEQ ID NO: 172 - protein, 10 aa, Homo sapiens
KLLWGDIMEL

SEQ ID NO: 173 - protein, 9 aa, Homo sapiens
KMQETLVGL

SEQ ID NO: 174 - protein, 9 aa, Homo sapiens
NLTENLQYV

SEQ ID NO: 175 - protein, 10 aa, Homo sapiens
KMDSFLDMQL

SEQ ID NO: 176 - protein, 9 aa, Homo sapiens
HLWTGEEQL

SEQ ID NO: 177 - protein, 9 aa, Homo sapiens
KITTVIQHV

SEQ ID NO: 178 - protein, 9 aa, Homo sapiens
KLWPLFVKL

SEQ ID NO: 179 - protein, 9 aa, Homo sapiens
RLISTLENL

SEQ ID NO: 180 - protein, 9 aa, Homo sapiens
ALDQEIIEV

SEQ ID NO: 181 - protein, 9 aa, Homo sapiens
KLLNHVTQL

SEQ ID NO: 182 - protein, 9 aa, Homo sapiens
SLSEYDQCL

SEQ ID NO: 183 - protein, 9 aa, Homo sapiens
SVIGVSPAV

SEQ ID NO: 184 - protein, 11 aa, Homo sapiens
RMTDQEAIQDL

SEQ ID NO: 185 - protein, 9 aa, Homo sapiens
RLIPIIVLL

SEQ ID NO: 186 - protein, 9 aa, Homo sapiens
IILDEAHNV

SEQ ID NO: 187 - protein, 9 aa, Homo sapiens
MLPPPPLTA

SEQ ID NO: 188 - protein, 9 aa, Homo sapiens
RLLDFPTLL

SEQ ID NO: 189 - protein, 9 aa, Homo sapiens
RLFEEVLGV

SEQ ID NO: 190 - protein, 9 aa, Homo sapiens
SLYKGLLSV

SEQ ID NO: 191 - protein, 9 aa, Homo sapiens
ALSVLRLAL

SEQ ID NO: 192 - protein, 9 aa, Homo sapiens
GLAALAVHL

SEQ ID NO: 193 - protein, 9 aa, Homo sapiens
FLLAEDTKV

SEQ ID NO: 194 - protein, 9 aa, Homo sapiens
LLWGNLPEI

SEQ ID NO: 195 - protein, 9 aa, Homo sapiens
FLFVDPELV

SEQ ID NO: 196 - protein, 9 aa, Homo sapiens
ILVDWLVQV

SEQ ID NO: 197 - protein, 10 aa, Homo sapiens
VLLNEILEQV

SEQ ID NO: 198 - protein, 9 aa, Homo sapiens
KIQEILTQV

SEQ ID NO: 199 - protein, 10 aa, Homo sapiens
ELAGIGILTV

SEQ ID NO: 200 - protein, 9 aa, Homo sapiens
YLLPAIVHI